European Patent Application EP 4 403 623 A1, published July 24, 2024. Title: Microalgae strain having an effect of promoting plant growth and use thereof. Applicant: 씨제이제일제당 (주). Application KR. The sequence listing filed with the application follows.

SEQUENCE LISTING (3 sequences)

SEQ ID NO: 1 - DNA, 1565 bp, synthetic construct
  misc_feature 1..1565: note = 18S rRNA sequence of Chlorella vulgaris CD02-3002 strain
  source 1..1565: mol_type = other DNA
tcgacttcctggaagggacgtatttattagataaaaggccgaccgggctctgcccgactcgcggtgaatcatgataacttcacgaatcgcatggccttgtgccggcgatgtttcattcaaatttctgccctatcaactttcgatggtaggatagaggcctaccatggtggtaacgggtgacggaggattagggttcgattccggagagggagcctgagaaacggctaccacatccaaggaaggcagcaggcgcgcaaattacccaatcctgacacagggaggtagtgacaataaataacaatactgggccttttcaggtctggtaattggaatgagtacaatctaaaccccttaacgaggatcaattggagggcaagtctggtgccagcagccgcggtaattccagctccaatagcgtatatttaagttgctgcagttaaaaagctcgtagttggatttcgggtggggcctgccggtccgccgtttcggtgtgcactggcagggcccaccttgttgccggggacgggctcctgggcttcactgtccgggactcggagtcggcgctgttactttgagtaaattagagtgttcaaagcaggcctacgctctgaatacattagcatggaataacacgataggactctggcctatcctgttggtctgtaggaccggagtaatgattaagagggacagtcgggggcattcgtatttcattgtcagaggtgaaattcttggatttatgaaagacgaactactgcgaaagcatttgccaaggatgttttcattaatcaagaacgaaagttgggggctcgaagacgattagataccgtcctagtctcaaccataaacgatgccgactagggatcggcggatgtttcttcgatgactccgccggcaccttatgagaaatcaaagtttttgggttccggggggagtatggtcgcaaggctgaaacttaaaggaattgacggaagggcaccaccaggcgtggagcctgcggcttaatttgactcaacacgggaaaacttaccaggtccagacatagtgaggattgacagattgagagctctttcttgattctatgggtggtggtgcatggccgttcttagttggtgggttgccttgtcaggttgattccggtaacgaacgagacctcagcctgctaaatagtcacggttggttctccagccggcggacttcttagagggactattggcgactagccaatggaagcatgaggcaataacaggtctgtgatgcccttagatgttctgggccgcacgcgcgctacactgatgcattcaacgagcctagccttggccgagaggcccgggtaatctttgaaactgcatcgtgatggggatagattattgcaattattaatcttcaacgaggaatgcctagtaagcgcaagtcatcagcttgcgttgattacgtccctgccctttgtacacaccgcccgtcgctcctaccgattgggtgtgctggtgaagtgttcggattggcgaccgggtgcggtctccgctctcggccgccgagaagttcattaaaccctcccacctaga

SEQ ID NO: 2 - DNA, 20 bp, synthetic construct
  misc_feature 1..20: note = 18s-F_primer
  source 1..20: mol_type = other DNA
cgacttctggaagggacgta

SEQ ID NO: 3 - DNA, 20 bp, synthetic construct
  misc_feature 1..20: note = 18s-R_primer
  source 1..20: mol_type = other DNA
ctaggtgggagggtttaatg